European Patent Specification EP 3 018 123 B1, published May 10, 2023. Title: Amide compound. Applicant: TAKEDA PHARMACEUTICAL COMPANY LIMITED. The sequence listing filed with the application follows.

SEQUENCE LISTING (1 sequence)

SEQ ID NO: 1 - protein, 20 aa, Artificial Sequence
CLTARHKILHRLLQEGSPSD